European Patent Application EP 4 549 548 A1, published May 7, 2025. Title: SYMBIOTIC BACTERIUM IN HUMANS FOR PROMOTING HAIR GROWTH AND USE THEREOF. Applicant: SHANGHAI MICROH THERAPEUTICS, LLC. Application CN PCT/CN2023/101022, filed June 19, 2023. The sequence listing filed with the application follows.

SEQUENCE LISTING (1 sequence)

SEQ ID NO: 1 - DNA, 1421 bp, synthetic construct
  source 1..1421: mol_type = other DNA
tgcagtcgagcgaacagacgaggagcttgctcctttgacgttagcggcggacgggtgagtaacacgtaggtaacctacctataagactgggataacttcgggaaaccggagctaataccggataatatttcgaaccgcatggttcgatagtgaaagatggctttgctatcacttatagatggacctgcgccgtattagctagttggtaaggtaacggcttaccaaggcaacgatacgtagccgacctgagagggtgatcggccacactggaactgagacacggtccagactcctacgggaggcagcagtagggaatcttccgcaatgggcgaaagcctgacggagcaacgccgcgtgagtgatgaaggtcttcggatcgtaaaactctgttattagggaagaacaaacgtgtaagtaactgtgcacgtcttgacggtacctaatcagaaagccacggctaactacgtgccagcagccgcggtaatacgtaggtggcaagcgttatccggaattattgggcgtaaagcgcgcgtaggcggttttttaagtctgatgtgaaagcccacggctcaaccgtggagggtcattggaaactggaaaacttgagtgcagaagaggaaagtggaattccatgtgtagcggtgaaatgcgcagagatatggaggaacaccagtggcgaaggcgactttctggtctgtaactgacgctgatgtgcgaaagcgtggggatcaaacaggattagataccctggtagtccacgccgtaaacgatgagtgctaagtgttagggggtttccgccccttagtgctgcagctaacgcattaagcactccgcctggggagtacgaccgcaaggttgaaactcaaaggaattgacggggacccgcacaagcggtggagcatgtggtttaattcgaagcaacgcgaagaaccttaccaaatcttgacatcctttgacccttctagagatagaagtttccccttcgggggacaaagtgacaggtggtgcatggttgtcgtcagctcgtgtcgtgagatgttgggttaagtcccgcaacgagcgcaacccttaagcttagttgccatcattaagttgggcactctaagttgactgccggtgacaaaccggaggaaggtggggatgacgtcaaatcatcatgccccttatgatttgggctacacacgtgctacaatggacaatacaaagggcagcgaaaccgcgaggtcaagcaaatcccataaagttgttctcagttcggattgtagtctgcaactcgactacatgaagctggaatcgctagtaatcgtagatcagcatgctacggtgaatacgttcccgggtcttgtacacaccgcccgtcacaccacgagagtttgtaacacccgaagccggtggagtaaccatttggagctagccgtcga